European Patent Specification EP 3 850 004 B1, published February 18, 2026. Title: NATURAL KILLER CELL COMPOSITIONS AND IMMUNOTHERAPY METHODS FOR TREATING HEPATOCELLULAR CARCINOMA. Applicant: Nkarta, Inc. The sequence listing filed with the application follows.

SEQUENCE LISTING (44 sequences)

SEQ ID NO: 1 - DNA, 1714 bp, Homo sapiens
  misc_feature: NK45-1 DNA
atggccttaccagtgaccgccttgctcctgccgctggccttgctgctccacgccgccaggccgttattcaaccaagaagttcaaattcccttgaccgaaagttactgtggcccatgtcctaaaaactggatatgttacaaaaataactgctaccaattttttgatgagagtaaaaactggtatgagagccaggcttcttgtatgtctcaaaatgccagccttctgaaagtatacagcaaagaggaccaggatttacttaaactggtgaagtcatatcattggatgggactagtacacattccaacaaatggatcttggcagtgggaagatggctccattctctcacccaacctactaacaataattgaaatgcagaagggagactgtgcactctatgcctcgagctttaaaggctatatagaaaactgttcaactccaaatacgtacatctgcatgcaaaggactgtggagtccaaatatggtcccccatgcccatcatgcccaatctacatctgggcgcccttggccgggacttgtggggtccttctcctgtcactggttatcaccctttactgcaaacggggcagaaagaaactcctgtatatattcaaacaaccatttatgagaccagtacaaactactcaagaggaagatggctgtagctgccgatttccagaagaagaagaaggaggatgtgaactgagagtgaagttcagcaggagcgcagacgcccccgcgtaccagcagggccagaaccagctctataacgagctcaatctaggacgaagagaggagtacgatgttttggacaagagacgtggccgggaccctgagatggggggaaagccgagaaggaagaaccctcaggaaggcctgtacaatgaactgcagaaagataagatggcggaggcctacagtgagattgggatgaaaggcgagcgccggaggggcaaggggcacgatggcctttaccagggtctcagtacagccaccaaggacacctacgacgcccttcacatgcaggccctgccccctcgcggctctggcgagggaaggggttccctgcttacttgcggcgacgtcgaagagaatcccggtccgatggccctcccagtaactgccctccttttgcccctcgcactccttcttcatgccgctcgccccaactgggtcaacgtgattagcgatttgaagaaaatcgaggaccttatacagtctatgcatattgacgctacactgtatactgagagtgatgtacacccgtcctgtaaggtaacggccatgaaatgctttcttctggagctccaggtcatcagcttggagtctggggacgcaagcatccacgatacggttgaaaacctcatcatccttgcgaacaactctctctcatctaatggaaacgttacagagagtgggtgtaaggagtgcgaagagttggaagaaaaaaacatcaaagaatttcttcaatccttcgttcacatagtgcaaatgttcattaacacgtccactaccacacccgccccgaggccacctacgccggcaccgactatcgccagtcaacccctctctctgcgccccgaggcttgccggcctgcggctggtggggcggtccacacccggggcctggattttgcgtgcgatatatacatctgggcacctcttgccggcacctgcggagtgctgcttctctcactcgttattacgctgtactgct

SEQ ID NO: 2 - protein, 571 aa, Homo sapiens
  MISC_FEATURE: NK45-1 Amino Acid
MALPVTALLLPLALLLHAARPLFNQEVQIPLTESYCGPCPKNWICYKNNCYQFFDESKNWYESQASCMSQNASLLKVYSKEDQDLLKLVKSYHWMGLVHIPTNGSWQWEDGSILSPNLLTIIEMQKGDCALYASSFKGYIENCSTPNTYICMQRTVESKYGPPCPSCPIYIWAPLAGTCGVLLLSLVITLYCKRGRKKLLYIFKQPFMRPVQTTQEEDGCSCRFPEEEEGGCELRVKFSRSADAPAYQQGQNQLYNELNLGRREEYDVLDKRRGRDPEMGGKPRRKNPQEGLYNELQKDKMAEAYSEIGMKGERRRGKGHDGLYQGLSTATKDTYDALHMQALPPRGSGEGRGSLLTCGDVEENPGPMALPVTALLLPLALLLHAARPNWVNVISDLKKIEDLIQSMHIDATLYTESDVHPSCKVTAMKCFLLELQVISLESGDASIHDTVENLIILANNSLSSNGNVTESGCKECEELEEKNIKEFLQSFVHIVQMFINTSTTTPAPRPPTPAPTIASQPLSLRPEACRPAAGGAVHTRGLDFACDIYIWAPLAGTCGVLLLSLVITLYC

SEQ ID NO: 3 - DNA, 1818 bp, Homo sapiens
  misc_feature: NK45-2 DNA
atggccttaccagtgaccgccttgctcctgccgctggccttgctgctccacgccgccaggccgttattcaaccaagaagttcaaattcccttgaccgaaagttactgtggcccatgtcctaaaaactggatatgttacaaaaataactgctaccaattttttgatgagagtaaaaactggtatgagagccaggcttcttgtatgtctcaaaatgccagccttctgaaagtatacagcaaagaggaccaggatttacttaaactggtgaagtcatatcattggatgggactagtacacattccaacaaatggatcttggcagtgggaagatggctccattctctcacccaacctactaacaataattgaaatgcagaagggagactgtgcactctatgcctcgagctttaaaggctatatagaaaactgttcaactccaaatacgtacatctgcatgcaaaggactgtgaccacgacgccagcgccgcgaccaccaacaccggcgcccaccatcgcgtcgcagcccctgtccctgcgcccagaggcgtgccggccagcggcggggggcgcagtgcacacgagggggctggacttcgcctgtgatttttgggtgctggtggtggttggtggagtcctggcttgctatagcttgctagtaacagtggcctttattattttctgggtgaggagtaagaggagcaggctcctgcacagtgactacatgaacatgactccccgccgccccgggcccacccgcaagcattaccagccctatgccccaccacgcgacttcgcagcctatcgctccagagtgaagttcagcaggagcgcagacgcccccgcgtaccagcagggccagaaccagctctataacgagctcaatctaggacgaagagaggagtacgatgttttggacaagagacgtggccgggaccctgagatggggggaaagccgagaaggaagaaccctcaggaaggcctgtacaatgaactgcagaaagataagatggcggaggcctacagtgagattgggatgaaaggcgagcgccggaggggcaaggggcacgatggcctttaccagggtctcagtacagccaccaaggacacctacgacgcccttcacatgcaggccctgccccctcgcggctctggcgagggaaggggttccctgcttacttgcggcgacgtcgaagagaatcccggtccgatggccctcccagtaactgccctccttttgcccctcgcactccttcttcatgccgctcgccccaactgggtcaacgtgattagcgatttgaagaaaatcgaggaccttatacagtctatgcatattgacgctacactgtatactgagagtgatgtacacccgtcctgtaaggtaacggccatgaaatgctttcttctggagctccaggtcatcagcttggagtctggggacgcaagcatccacgatacggttgaaaacctcatcatccttgcgaacaactctctctcatctaatggaaacgttacagagagtgggtgtaaggagtgcgaagagttggaagaaaaaaacatcaaagaatttcttcaatccttcgttcacatagtgcaaatgttcattaacacgtccactaccacacccgccccgaggccacctacgccggcaccgactatcgccagtcaacccctctctctgcgccccgaggcttgccggcctgcggctggtggggcggtccacacccggggcctggattttgcgtgcgatatatacatctgggcacctcttgccggcacctgcggagtgctgcttctctcactcgttattacgctgtactgc

SEQ ID NO: 4 - protein, 606 aa, Homo sapiens
  MISC_FEATURE: NK45-2 Amino Acid
MALPVTALLLPLALLLHAARPLFNQEVQIPLTESYCGPCPKNWICYKNNCYQFFDESKNWYESQASCMSQNASLLKVYSKEDQDLLKLVKSYHWMGLVHIPTNGSWQWEDGSILSPNLLTIIEMQKGDCALYASSFKGYIENCSTPNTYICMQRTVTTTPAPRPPTPAPTIASQPLSLRPEACRPAAGGAVHTRGLDFACDFWVLVVVGGVLACYSLLVTVAFIIFWVRSKRSRLLHSDYMNMTPRRPGPTRKHYQPYAPPRDFAAYRSRVKFSRSADAPAYQQGQNQLYNELNLGRREEYDVLDKRRGRDPEMGGKPRRKNPQEGLYNELQKDKMAEAYSEIGMKGERRRGKGHDGLYQGLSTATKDTYDALHMQALPPRGSGEGRGSLLTCGDVEENPGPMALPVTALLLPLALLLHAARPNWVNVISDLKKIEDLIQSMHIDATLYTESDVHPSCKVTAMKCFLLELQVISLESGDASIHDTVENLIILANNSLSSNGNVTESGCKECEELEEKNIKEFLQSFVHIVQMFINTSTTTPAPRPPTPAPTIASQPLSLRPEACRPAAGGAVHTRGLDFACDIYIWAPLAGTCGVLLLSLVITLYC

SEQ ID NO: 5 - DNA, 1719 bp, Homo sapiens
  misc_feature: NK45-3 DNA
atggccttaccagtgaccgccttgctcctgccgctggccttgctgctccacgccgccaggccgttattcaaccaagaagttcaaattcccttgaccgaaagttactgtggcccatgtcctaaaaactggatatgttacaaaaataactgctaccaattttttgatgagagtaaaaactggtatgagagccaggcttcttgtatgtctcaaaatgccagccttctgaaagtatacagcaaagaggaccaggatttacttaaactggtgaagtcatatcattggatgggactagtacacattccaacaaatggatcttggcagtgggaagatggctccattctctcacccaacctactaacaataattgaaatgcagaagggagactgtgcactctatgcctcgagctttaaaggctatatagaaaactgttcaactccaaatacgtacatctgcatgcaaaggactgtggagtccaaatatggtcccccatgcccatcatgcccattttgggtgctggtggtggttggtggagtcctggcttgctatagcttgctagtaacagtggcctttattattttctgggtgaggagtaagaggagcaggctcctgcacagtgactacatgaacatgactccccgccgccccgggcccacccgcaagcattaccagccctatgccccaccacgcgacttcgcagcctatcgctccagagtgaagttcagcaggagcgcagacgcccccgcgtaccagcagggccagaaccagctctataacgagctcaatctaggacgaagagaggagtacgatgttttggacaagagacgtggccgggaccctgagatggggggaaagccgagaaggaagaaccctcaggaaggcctgtacaatgaactgcagaaagataagatggcggaggcctacagtgagattgggatgaaaggcgagcgccggaggggcaaggggcacgatggcctttaccagggtctcagtacagccaccaaggacacctacgacgcccttcacatgcaggccctgccccctcgcggctctggcgagggaaggggttccctgcttacttgcggcgacgtcgaagagaatcccggtccgatggccctcccagtaactgccctccttttgcccctcgcactccttcttcatgccgctcgccccaactgggtcaacgtgattagcgatttgaagaaaatcgaggaccttatacagtctatgcatattgacgctacactgtatactgagagtgatgtacacccgtcctgtaaggtaacggccatgaaatgctttcttctggagctccaggtcatcagcttggagtctggggacgcaagcatccacgatacggttgaaaacctcatcatccttgcgaacaactctctctcatctaatggaaacgttacagagagtgggtgtaaggagtgcgaagagttggaagaaaaaaacatcaaagaatttcttcaatccttcgttcacatagtgcaaatgttcattaacacgtccactaccacacccgccccgaggccacctacgccggcaccgactatcgccagtcaacccctctctctgcgccccgaggcttgccggcctgcggctggtggggcggtccacacccggggcctggattttgcgtgcgatatatacatctgggcacctcttgccggcacctgcggagtgctgcttctctcactcgttattacgctgtactgc

SEQ ID NO: 6 - protein, 573 aa, Homo sapiens
  MISC_FEATURE: NK45-3 Amino Acid
MALPVTALLLPLALLLHAARPLFNQEVQIPLTESYCGPCPKNWICYKNNCYQFFDESKNWYESQASCMSQNASLLKVYSKEDQDLLKLVKSYHWMGLVHIPTNGSWQWEDGSILSPNLLTIIEMQKGDCALYASSFKGYIENCSTPNTYICMQRTVESKYGPPCPSCPFWVLVVVGGVLACYSLLVTVAFIIFWVRSKRSRLLHSDYMNMTPRRPGPTRKHYQPYAPPRDFAAYRSRVKFSRSADAPAYQQGQNQLYNELNLGRREEYDVLDKRRGRDPEMGGKPRRKNPQEGLYNELQKDKMAEAYSEIGMKGERRRGKGHDGLYQGLSTATKDTYDALHMQALPPRGSGEGRGSLLTCGDVEENPGPMALPVTALLLPLALLLHAARPNWVNVISDLKKIEDLIQSMHIDATLYTESDVHPSCKVTAMKCFLLELQVISLESGDASIHDTVENLIILANNSLSSNGNVTESGCKECEELEEKNIKEFLQSFVHIVQMFINTSTTTPAPRPPTPAPTIASQPLSLRPEACRPAAGGAVHTRGLDFACDIYIWAPLAGTCGVLLLSLVITLYC

SEQ ID NO: 7 - DNA, 1797 bp, Homo sapiens
  misc_feature: NK45-4 DNA
atggccttaccagtgaccgccttgctcctgccgctggccttgctgctccacgccgccaggccgttattcaaccaagaagttcaaattcccttgaccgaaagttactgtggcccatgtcctaaaaactggatatgttacaaaaataactgctaccaattttttgatgagagtaaaaactggtatgagagccaggcttcttgtatgtctcaaaatgccagccttctgaaagtatacagcaaagaggaccaggatttacttaaactggtgaagtcatatcattggatgggactagtacacattccaacaaatggatcttggcagtgggaagatggctccattctctcacccaacctactaacaataattgaaatgcagaagggagactgtgcactctatgcctcgagctttaaaggctatatagaaaactgttcaactccaaatacgtacatctgcatgcaaaggactgtgaccacgacgccagcgccgcgaccaccaacaccggcgcccaccatcgcgtcgcagcccctgtccctgcgcccagaggcgtgccggccagcggcggggggcgcagtgcacacgagggggctggacttcgcctgtgatatctacatctgggcgcccttggccgggacttgtggggtccttctcctgtcactggttatcaccctttactgccggagggaccagaggctgccccccgatgcccacaagccccctgggggaggcagtttccggacccccatccaagaggagcaggccgacgcccactccaccctggccaagatcagagtgaagttcagcaggagcgcagacgcccccgcgtaccagcagggccagaaccagctctataacgagctcaatctaggacgaagagaggagtacgatgttttggacaagagacgtggccgggaccctgagatggggggaaagccgagaaggaagaaccctcaggaaggcctgtacaatgaactgcagaaagataagatggcggaggcctacagtgagattgggatgaaaggcgagcgccggaggggcaaggggcacgatggcctttaccagggtctcagtacagccaccaaggacacctacgacgcccttcacatgcaggccctgccccctcgcggctctggcgagggaaggggttccctgcttacttgcggcgacgtcgaagagaatcccggtccgatggccctcccagtaactgccctccttttgcccctcgcactccttcttcatgccgctcgccccaactgggtcaacgtgattagcgatttgaagaaaatcgaggaccttatacagtctatgcatattgacgctacactgtatactgagagtgatgtacacccgtcctgtaaggtaacggccatgaaatgctttcttctggagctccaggtcatcagcttggagtctggggacgcaagcatccacgatacggttgaaaacctcatcatccttgcgaacaactctctctcatctaatggaaacgttacagagagtgggtgtaaggagtgcgaagagttggaagaaaaaaacatcaaagaatttcttcaatccttcgttcacatagtgcaaatgttcattaacacgtccactaccacacccgccccgaggccacctacgccggcaccgactatcgccagtcaacccctctctctgcgccccgaggcttgccggcctgcggctggtggggcggtccacacccggggcctggattttgcgtgcgatatatacatctgggcacctcttgccggcacctgcggagtgctgcttctctcactcgttattacgctgtactgc

SEQ ID NO: 8 - protein, 599 aa, Homo sapiens
  MISC_FEATURE: NK45-4 Amino Acid
MALPVTALLLPLALLLHAARPLFNQEVQIPLTESYCGPCPKNWICYKNNCYQFFDESKNWYESQASCMSQNASLLKVYSKEDQDLLKLVKSYHWMGLVHIPTNGSWQWEDGSILSPNLLTIIEMQKGDCALYASSFKGYIENCSTPNTYICMQRTVTTTPAPRPPTPAPTIASQPLSLRPEACRPAAGGAVHTRGLDFACDIYIWAPLAGTCGVLLLSLVITLYCRRDQRLPPDAHKPPGGGSFRTPIQEEQADAHSTLAKIRVKFSRSADAPAYQQGQNQLYNELNLGRREEYDVLDKRRGRDPEMGGKPRRKNPQEGLYNELQKDKMAEAYSEIGMKGERRRGKGHDGLYQGLSTATKDTYDALHMQALPPRGSGEGRGSLLTCGDVEENPGPMALPVTALLLPLALLLHAARPNWVNVISDLKKIEDLIQSMHIDATLYTESDVHPSCKVTAMKCFLLELQVISLESGDASIHDTVENLIILANNSLSSNGNVTESGCKECEELEEKNIKEFLQSFVHIVQMFINTSTTTPAPRPPTPAPTIASQPLSLRPEACRPAAGGAVHTRGLDFACDIYIWAPLAGTCGVLLLSLVITLYC

SEQ ID NO: 9 - DNA, 1698 bp, Homo sapiens
  misc_feature: NK45-5 DNA
atggccttaccagtgaccgccttgctcctgccgctggccttgctgctccacgccgccaggccgttattcaaccaagaagttcaaattcccttgaccgaaagttactgtggcccatgtcctaaaaactggatatgttacaaaaataactgctaccaattttttgatgagagtaaaaactggtatgagagccaggcttcttgtatgtctcaaaatgccagccttctgaaagtatacagcaaagaggaccaggatttacttaaactggtgaagtcatatcattggatgggactagtacacattccaacaaatggatcttggcagtgggaagatggctccattctctcacccaacctactaacaataattgaaatgcagaagggagactgtgcactctatgcctcgagctttaaaggctatatagaaaactgttcaactccaaatacgtacatctgcatgcaaaggactgtggagtccaaatatggtcccccatgcccatcatgcccaatctacatctgggcgcccttggccgggacttgtggggtccttctcctgtcactggttatcaccctttactgccggagggaccagaggctgccccccgatgcccacaagccccctgggggaggcagtttccggacccccatccaagaggagcaggccgacgcccactccaccctggccaagatcagagtgaagttcagcaggagcgcagacgcccccgcgtaccagcagggccagaaccagctctataacgagctcaatctaggacgaagagaggagtacgatgttttggacaagagacgtggccgggaccctgagatggggggaaagccgagaaggaagaaccctcaggaaggcctgtacaatgaactgcagaaagataagatggcggaggcctacagtgagattgggatgaaaggcgagcgccggaggggcaaggggcacgatggcctttaccagggtctcagtacagccaccaaggacacctacgacgcccttcacatgcaggccctgccccctcgcggctctggcgagggaaggggttccctgcttacttgcggcgacgtcgaagagaatcccggtccgatggccctcccagtaactgccctccttttgcccctcgcactccttcttcatgccgctcgccccaactgggtcaacgtgattagcgatttgaagaaaatcgaggaccttatacagtctatgcatattgacgctacactgtatactgagagtgatgtacacccgtcctgtaaggtaacggccatgaaatgctttcttctggagctccaggtcatcagcttggagtctggggacgcaagcatccacgatacggttgaaaacctcatcatccttgcgaacaactctctctcatctaatggaaacgttacagagagtgggtgtaaggagtgcgaagagttggaagaaaaaaacatcaaagaatttcttcaatccttcgttcacatagtgcaaatgttcattaacacgtccactaccacacccgccccgaggccacctacgccggcaccgactatcgccagtcaacccctctctctgcgccccgaggcttgccggcctgcggctggtggggcggtccacacccggggcctggattttgcgtgcgatatatacatctgggcacctcttgccggcacctgcggagtgctgcttctctcactcgttattacgctgtactgc

SEQ ID NO: 10 - protein, 566 aa, Homo sapiens
  MISC_FEATURE: NK45-5 Amino Acid
MALPVTALLLPLALLLHAARPLFNQEVQIPLTESYCGPCPKNWICYKNNCYQFFDESKNWYESQASCMSQNASLLKVYSKEDQDLLKLVKSYHWMGLVHIPTNGSWQWEDGSILSPNLLTIIEMQKGDCALYASSFKGYIENCSTPNTYICMQRTVESKYGPPCPSCPIYIWAPLAGTCGVLLLSLVITLYCRRDQRLPPDAHKPPGGGSFRTPIQEEQADAHSTLAKIRVKFSRSADAPAYQQGQNQLYNELNLGRREEYDVLDKRRGRDPEMGGKPRRKNPQEGLYNELQKDKMAEAYSEIGMKGERRRGKGHDGLYQGLSTATKDTYDALHMQALPPRGSGEGRGSLLTCGDVEENPGPMALPVTALLLPLALLLHAARPNWVNVISDLKKIEDLIQSMHIDATLYTESDVHPSCKVTAMKCFLLELQVISLESGDASIHDTVENLIILANNSLSSNGNVTESGCKECEELEEKNIKEFLQSFVHIVQMFINTSTTTPAPRPPTPAPTIASQPLSLRPEACRPAAGGAVHTRGLDFACDIYIWAPLAGTCGVLLLSLVITLYC

SEQ ID NO: 11 - DNA, 1800 bp, Homo sapiens
  misc_feature: NK45-6 DNA
atggccttaccagtgaccgccttgctcctgccgctggccttgctgctccacgccgccaggccgttattcaaccaagaagttcaaattcccttgaccgaaagttactgtggcccatgtcctaaaaactggatatgttacaaaaataactgctaccaattttttgatgagagtaaaaactggtatgagagccaggcttcttgtatgtctcaaaatgccagccttctgaaagtatacagcaaagaggaccaggatttacttaaactggtgaagtcatatcattggatgggactagtacacattccaacaaatggatcttggcagtgggaagatggctccattctctcacccaacctactaacaataattgaaatgcagaagggagactgtgcactctatgcctcgagctttaaaggctatatagaaaactgttcaactccaaatacgtacatctgcatgcaaaggactgtgaccacgacgccagcgccgcgaccaccaacaccggcgcccaccatcgcgtcgcagcccctgtccctgcgcccagaggcgtgccggccagcggcggggggcgcagtgcacacgagggggctggacttcgcctgtgatcccaaactctgctacctgctggatggaatcctcttcatctatggtgtcattctcactgccttgttcctgaagaggagcaggctcctgcacagtgactacatgaacatgactccccgccgccccgggcccacccgcaagcattaccagccctatgccccaccacgcgacttcgcagcctatcgctccagagtgaagttcagcaggagcgcagacgcccccgcgtaccagcagggccagaaccagctctataacgagctcaatctaggacgaagagaggagtacgatgttttggacaagagacgtggccgggaccctgagatggggggaaagccgagaaggaagaaccctcaggaaggcctgtacaatgaactgcagaaagataagatggcggaggcctacagtgagattgggatgaaaggcgagcgccggaggggcaaggggcacgatggcctttaccagggtctcagtacagccaccaaggacacctacgacgcccttcacatgcaggccctgccccctcgcggctctggcgagggaaggggttccctgcttacttgcggcgacgtcgaagagaatcccggtccgatggccctcccagtaactgccctccttttgcccctcgcactccttcttcatgccgctcgccccaactgggtcaacgtgattagcgatttgaagaaaatcgaggaccttatacagtctatgcatattgacgctacactgtatactgagagtgatgtacacccgtcctgtaaggtaacggccatgaaatgctttcttctggagctccaggtcatcagcttggagtctggggacgcaagcatccacgatacggttgaaaacctcatcatccttgcgaacaactctctctcatctaatggaaacgttacagagagtgggtgtaaggagtgcgaagagttggaagaaaaaaacatcaaagaatttcttcaatccttcgttcacatagtgcaaatgttcattaacacgtccactaccacacccgccccgaggccacctacgccggcaccgactatcgccagtcaacccctctctctgcgccccgaggcttgccggcctgcggctggtggggcggtccacacccggggcctggattttgcgtgcgatatatacatctgggcacctcttgccggcacctgcggagtgctgcttctctcactcgttattacgctgtactgc

SEQ ID NO: 12 - protein, 600 aa, Homo sapiens
  MISC_FEATURE: NK45-6 Amino Acid
MALPVTALLLPLALLLHAARPLFNQEVQIPLTESYCGPCPKNWICYKNNCYQFFDESKNWYESQASCMSQNASLLKVYSKEDQDLLKLVKSYHWMGLVHIPTNGSWQWEDGSILSPNLLTIIEMQKGDCALYASSFKGYIENCSTPNTYICMQRTVTTTPAPRPPTPAPTIASQPLSLRPEACRPAAGGAVHTRGLDFACDPKLCYLLDGILFIYGVILTALFLKRSRLLHSDYMNMTPRRPGPTRKHYQPYAPPRDFAAYRSRVKFSRSADAPAYQQGQNQLYNELNLGRREEYDVLDKRRGRDPEMGGKPRRKNPQEGLYNELQKDKMAEAYSEIGMKGERRRGKGHDGLYQGLSTATKDTYDALHMQALPPRGSGEGRGSLLTCGDVEENPGPMALPVTALLLPLALLLHAARPNWVNVISDLKKIEDLIQSMHIDATLYTESDVHPSCKVTAMKCFLLELQVISLESGDASIHDTVENLIILANNSLSSNGNVTESGCKECEELEEKNIKEFLQSFVHIVQMFINTSTTTPAPRPPTPAPTIASQPLSLRPEACRPAAGGAVHTRGLDFACDIYIWAPLAGTCGVLLLSLVITLYC

SEQ ID NO: 13 - DNA, 1944 bp, Homo sapiens
  misc_feature: NK45-7 DNA
atggccttaccagtgaccgccttgctcctgccgctggccttgctgctccacgccgccaggccgttattcaaccaagaagttcaaattcccttgaccgaaagttactgtggcccatgtcctaaaaactggatatgttacaaaaataactgctaccaattttttgatgagagtaaaaactggtatgagagccaggcttcttgtatgtctcaaaatgccagccttctgaaagtatacagcaaagaggaccaggatttacttaaactggtgaagtcatatcattggatgggactagtacacattccaacaaatggatcttggcagtgggaagatggctccattctctcacccaacctactaacaataattgaaatgcagaagggagactgtgcactctatgcctcgagctttaaaggctatatagaaaactgttcaactccaaatacgtacatctgcatgcaaaggactgtgaccacgacgccagcgccgcgaccaccaacaccggcgcccaccatcgcgtcgcagcccctgtccctgcgcccagaggcgtgccggccagcggcggggggcgcagtgcacacgagggggctggacttcgcctgtgatttttgggtgctggtggtggttggtggagtcctggcttgctatagcttgctagtaacagtggcctttattattttctgggtgaggagtaagaggagcaggctcctgcacagtgactacatgaacatgactccccgccgccccgggcccacccgcaagcattaccagccctatgccccaccacgcgacttcgcagcctatcgctccaaacggggcagaaagaaactcctgtatatattcaaacaaccatttatgagaccagtacaaactactcaagaggaagatggctgtagctgccgatttccagaagaagaagaaggaggatgtgaactgagagtgaagttcagcaggagcgcagacgcccccgcgtaccagcagggccagaaccagctctataacgagctcaatctaggacgaagagaggagtacgatgttttggacaagagacgtggccgggaccctgagatggggggaaagccgagaaggaagaaccctcaggaaggcctgtacaatgaactgcagaaagataagatggcggaggcctacagtgagattgggatgaaaggcgagcgccggaggggcaaggggcacgatggcctttaccagggtctcagtacagccaccaaggacacctacgacgcccttcacatgcaggccctgccccctcgcggctctggcgagggaaggggttccctgcttacttgcggcgacgtcgaagagaatcccggtccgatggccctcccagtaactgccctccttttgcccctcgcactccttcttcatgccgctcgccccaactgggtcaacgtgattagcgatttgaagaaaatcgaggaccttatacagtctatgcatattgacgctacactgtatactgagagtgatgtacacccgtcctgtaaggtaacggccatgaaatgctttcttctggagctccaggtcatcagcttggagtctggggacgcaagcatccacgatacggttgaaaacctcatcatccttgcgaacaactctctctcatctaatggaaacgttacagagagtgggtgtaaggagtgcgaagagttggaagaaaaaaacatcaaagaatttcttcaatccttcgttcacatagtgcaaatgttcattaacacgtccactaccacacccgccccgaggccacctacgccggcaccgactatcgccagtcaacccctctctctgcgccccgaggcttgccggcctgcggctggtggggcggtccacacccggggcctggattttgcgtgcgatatatacatctgggcacctcttgccggcacctgcggagtgctgcttctctcactcgttattacgctgtactgc

SEQ ID NO: 14 - protein, 648 aa, Homo sapiens
  MISC_FEATURE: NK45-7 Amino Acid
MALPVTALLLPLALLLHAARPLFNQEVQIPLTESYCGPCPKNWICYKNNCYQFFDESKNWYESQASCMSQNASLLKVYSKEDQDLLKLVKSYHWMGLVHIPTNGSWQWEDGSILSPNLLTIIEMQKGDCALYASSFKGYIENCSTPNTYICMQRTVTTTPAPRPPTPAPTIASQPLSLRPEACRPAAGGAVHTRGLDFACDFWVLVVVGGVLACYSLLVTVAFIIFWVRSKRSRLLHSDYMNMTPRRPGPTRKHYQPYAPPRDFAAYRSKRGRKKLLYIFKQPFMRPVQTTQEEDGCSCRFPEEEEGGCELRVKFSRSADAPAYQQGQNQLYNELNLGRREEYDVLDKRRGRDPEMGGKPRRKNPQEGLYNELQKDKMAEAYSEIGMKGERRRGKGHDGLYQGLSTATKDTYDALHMQALPPRGSGEGRGSLLTCGDVEENPGPMALPVTALLLPLALLLHAARPNWVNVISDLKKIEDLIQSMHIDATLYTESDVHPSCKVTAMKCFLLELQVISLESGDASIHDTVENLIILANNSLSSNGNVTESGCKECEELEEKNIKEFLQSFVHIVQMFINTSTTTPAPRPPTPAPTIASQPLSLRPEACRPAAGGAVHTRGLDFACDIYIWAPLAGTCGVLLLSLVITLYC

SEQ ID NO: 15 - DNA, 1812 bp, Homo sapiens
  misc_feature: NK26-8 DNA
atggccttaccagtgaccgccttgctcctgccgctggccttgctgctccacgccgccaggccgttattcaaccaagaagttcaaattcccttgaccgaaagttactgtggcccatgtcctaaaaactggatatgttacaaaaataactgctaccaattttttgatgagagtaaaaactggtatgagagccaggcttcttgtatgtctcaaaatgccagccttctgaaagtatacagcaaagaggaccaggatttacttaaactggtgaagtcatatcattggatgggactagtacacattccaacaaatggatcttggcagtgggaagatggctccattctctcacccaacctactaacaataattgaaatgcagaagggagactgtgcactctatgcctcgagctttaaaggctatatagaaaactgttcaactccaaatacgtacatctgcatgcaaaggactgtgaccacgacgccagcgccgcgaccaccaacaccggcgcccaccatcgcgtcgcagcccctgtccctgcgcccagaggcgtgccggccagcggcggggggcgcagtgcacacgagggggctggacttcgcctgtgatatctacatctgggcgcccttggccgggacttgtggggtccttctcctgtcactggttatcaccctttactgcaaacggggcagaaagaaactcctgtatatattcaaacaaccatttatgagaccagtacaaactactcaagaggaagatggctgtagctgccgatttccagaagaagaagaaggaggatgtgaactgagagtgaagttcagcaggagcgcagacgcccccgcgtaccagcagggccagaaccagctctataacgagctcaatctaggacgaagagaggagtacgatgttttggacaagagacgtggccgggaccctgagatggggggaaagccgagaaggaagaaccctcaggaaggcctgtacaatgaactgcagaaagataagatggcggaggcctacagtgagattgggatgaaaggcgagcgccggaggggcaaggggcacgatggcctttaccagggtctcagtacagccaccaaggacacctacgacgcccttcacatgcaggccctgccacctcgcggctctggcgagggaaggggttccctgcttacttgcggcgacgtcgaagagaatcccggtccgatggccctcccagtaactgccctccttttgcccctcgcactccttcttcatgccgctcgccccaactgggtcaacgtgattagcgatttgaagaaaatcgaggaccttatacagtctatgcatattgacgctacactgtatactgagagtgatgtacacccgtcctgtaaggtaacggccatgaaatgctttcttctggagctccaggtcatcagcttggagtctggggacgcaagcatccacgatacggttgaaaacctcatcatccttgcgaacaactctctctcatctaatggaaacgttacagagagtgggtgtaaggagtgcgaagagttggaagaaaaaaacatcaaagaatttcttcaatccttcgttcacatagtgcaaatgttcattaacacgtccactaccacacccgccccgaggccacctacgccggcaccgactatcgccagtcaacccctctctctgcgccccgaggcttgccggcctgcggctggtggggcggtccacacccggggcctggattttgcgtgcgatatatacatctgggcacctcttgccggcacctgcggagtgctgcttctctcactcgttattacgctgtactgc

SEQ ID NO: 16 - protein, 604 aa, Homo sapiens
  MISC_FEATURE: NK26-8 Amino Acid
MALPVTALLLPLALLLHAARPLFNQEVQIPLTESYCGPCPKNWICYKNNCYQFFDESKNWYESQASCMSQNASLLKVYSKEDQDLLKLVKSYHWMGLVHIPTNGSWQWEDGSILSPNLLTIIEMQKGDCALYASSFKGYIENCSTPNTYICMQRTVTTTPAPRPPTPAPTIASQPLSLRPEACRPAAGGAVHTRGLDFACDIYIWAPLAGTCGVLLLSLVITLYCKRGRKKLLYIFKQPFMRPVQTTQEEDGCSCRFPEEEEGGCELRVKFSRSADAPAYQQGQNQLYNELNLGRREEYDVLDKRRGRDPEMGGKPRRKNPQEGLYNELQKDKMAEAYSEIGMKGERRRGKGHDGLYQGLSTATKDTYDALHMQALPPRGSGEGRGSLLTCGDVEENPGPMALPVTALLLPLALLLHAARPNWVNVISDLKKIEDLIQSMHIDATLYTESDVHPSCKVTAMKCFLLELQVISLESGDASIHDTVENLIILANNSLSSNGNVTESGCKECEELEEKNIKEFLQSFVHIVQMFINTSTTTPAPRPPTPAPTIASQPLSLRPEACRPAAGGAVHTRGLDFACDIYIWAPLAGTCGVLLLSLVITLYC

SEQ ID NO: 17 - DNA, 1818 bp, Homo sapiens
atggctctgcccgtcaccgcactgctgctgcctctggctctgctgctgcacgccgcacgaccactgttcaatcaggaagtccagatccccctgacagagtcttactgcggcccatgtcccaagaactggatctgctacaagaacaattgttatcagttctttgacgagagcaagaactggtatgagtcccaggcctcttgcatgagccagaatgcctctctgctgaaggtgtacagcaaggaggaccaggatctgctgaagctggtgaagtcctatcactggatgggcctggtgcacatccctacaaacggctcttggcagtgggaggacggctccatcctgtctccaaatctgctgaccatcatcgagatgcagaagggcgattgcgccctgtacgccagctccttcaagggctatatcgagaactgctccacacccaatacctacatctgtatgcagaggaccgtgaccacaacccctgcaccacgcccccctacaccagcacctaccatcgcaagccagcctctgtccctgcggccagaggcatgtagaccagcagcaggaggagcagtgcacacaagaggcctggacttcgcctgcgatcccaaactctgctacctgctggatggaatcctcttcatctatggtgtcattctcactgccttgttcctgctttactgcaagcggggcagaaagaagctgctgtatatcttcaagcagcccttcatgcggcccgtgcagacaacccaggaggaagacggctgctcatgtagatttcctgaagaagaagaagggggctgtgaactgagagtgaagttcagcaggagcgcagacgcccccgcgtaccagcagggccagaaccagctctataacgagctcaatctaggacgaagagaggagtacgatgttttggacaagagacgtggccgggaccctgagatggggggaaagccgagaaggaagaaccctcaggaaggcctgtacaatgaactgcagaaagataagatggcggaggcctacagtgagattgggatgaaaggcgagcgccggaggggcaaggggcacgatggcctttaccagggtctcagtacagccaccaaggacacctacgacgcccttcacatgcaggccctgccccctcgcggctctggcgagggaaggggttccctgcttacttgcggcgacgtcgaagagaatcccggtccgatggccctcccagtaactgccctccttttgcccctcgcactccttcttcatgccgctcgccccaactgggtcaacgtgattagcgatttgaagaaaatcgaggaccttatacagtctatgcatattgacgctacactgtatactgagagtgatgtacacccgtcctgtaaggtaacggccatgaaatgctttcttctggagctccaggtcatcagcttggagtctggggacgcaagcatccacgatacggttgaaaacctcatcatccttgcgaacaactctctctcatctaatggaaacgttacagagagtgggtgtaaggagtgcgaagagttggaagaaaaaaacatcaaagaatttcttcaatccttcgttcacatagtgcaaatgttcattaacacgtccactaccacacccgccccgaggccacctacgccggcaccgactatcgccagtcaacccctctctctgcgccccgaggcttgccggcctgcggctggtggggcggtccacacccggggcctggattttgcgtgcgatatatacatctgggcacctcttgccggcacctgcggagtgctgcttctctcactcgttattacgctgtactgc

SEQ ID NO: 18 - protein, 606 aa, Homo sapiens
  MISC_FEATURE: NK39-5 Amino Acid
MALPVTALLLPLALLLHAARPLFNQEVQIPLTESYCGPCPKNWICYKNNCYQFFDESKNWYESQASCMSQNASLLKVYSKEDQDLLKLVKSYHWMGLVHIPTNGSWQWEDGSILSPNLLTIIEMQKGDCALYASSFKGYIENCSTPNTYICMQRTVTTTPAPRPPTPAPTIASQPLSLRPEACRPAAGGAVHTRGLDFACDPKLCYLLDGILFIYGVILTALFLLYCKRGRKKLLYIFKQPFMRPVQTTQEEDGCSCRFPEEEEGGCELRVKFSRSADAPAYQQGQNQLYNELNLGRREEYDVLDKRRGRDPEMGGKPRRKNPQEGLYNELQKDKMAEAYSEIGMKGERRRGKGHDGLYQGLSTATKDTYDALHMQALPPRGSGEGRGSLLTCGDVEENPGPMALPVTALLLPLALLLHAARPNWVNVISDLKKIEDLIQSMHIDATLYTESDVHPSCKVTAMKCFLLELQVISLESGDASIHDTVENLIILANNSLSSNGNVTESGCKECEELEEKNIKEFLQSFVHIVQMFINTSTTTPAPRPPTPAPTIASQPLSLRPEACRPAAGGAVHTRGLDFACDIYIWAPLAGTCGVLLLSLVITLYC

SEQ ID NO: 19 - DNA, 1641 bp, Homo sapiens
  misc_feature: NK39-6 DNA
atggctctgcccgtcaccgcactgctgctgcctctggctctgctgctgcacgccgcacgaccactgttcaatcaggaagtccagatccccctgacagagtcttactgcggcccatgtcccaagaactggatctgctacaagaacaattgttatcagttctttgacgagagcaagaactggtatgagtcccaggcctcttgcatgagccagaatgcctctctgctgaaggtgtacagcaaggaggaccaggatctgctgaagctggtgaagtcctatcactggatgggcctggtgcacatccctacaaacggctcttggcagtgggaggacggctccatcctgtctccaaatctgctgaccatcatcgagatgcagaagggcgattgcgccctgtacgccagctccttcaagggctatatcgagaactgctccacacccaatacctacatctgtatgcagaggaccgtgaccacaacccctgcaccacgcccccctacaccagcacctaccatcgcaagccagcctctgtccctgcggccagaggcatgtagaccagcagcaggaggagcagtgcacacaagaggcctggacttcgcctgcgatcccaaactctgctacctgctggatggaatcctcttcatctatggtgtcattctcactgccttgttcctgctttactgcaagcggggcagaaagaagctgctgtatatcttcaagcagcccttcatgcggcccgtgcagacaacccaggaggaagacggctgctcatgtagatttcctgaagaagaagaagggggctgtgaactgggcggaggaggcagcggcggcggcggcagcggcggcggcggcagcatgcaggatgaggacggctacatgaccctgaacgtgcagagcaagaagaggagcagcgcccagaccagccagctgaccttcaaggactacagcgtgaccctgcactggtacaagggctctggcgagggaaggggttccctgcttacttgcggcgacgtcgaagagaatcccggtccgatggccctcccagtaactgccctccttttgcccctcgcactccttcttcatgccgctcgccccaactgggtcaacgtgattagcgatttgaagaaaatcgaggaccttatacagtctatgcatattgacgctacactgtatactgagagtgatgtacacccgtcctgtaaggtaacggccatgaaatgctttcttctggagctccaggtcatcagcttggagtctggggacgcaagcatccacgatacggttgaaaacctcatcatccttgcgaacaactctctctcatctaatggaaacgttacagagagtgggtgtaaggagtgcgaagagttggaagaaaaaaacatcaaagaatttcttcaatccttcgttcacatagtgcaaatgttcattaacacgtccactaccacacccgccccgaggccacctacgccggcaccgactatcgccagtcaacccctctctctgcgccccgaggcttgccggcctgcggctggtggggcggtccacacccggggcctggattttgcgtgcgatatatacatctgggcacctcttgccggcacctgcggagtgctgcttctctcactcgttattacgctgtactgc

SEQ ID NO: 20 - protein, 547 aa, Homo sapiens
  MISC_FEATURE: NK39-6 Amino Acid
MALPVTALLLPLALLLHAARPLFNQEVQIPLTESYCGPCPKNWICYKNNCYQFFDESKNWYESQASCMSQNASLLKVYSKEDQDLLKLVKSYHWMGLVHIPTNGSWQWEDGSILSPNLLTIIEMQKGDCALYASSFKGYIENCSTPNTYICMQRTVTTTPAPRPPTPAPTIASQPLSLRPEACRPAAGGAVHTRGLDFACDPKLCYLLDGILFIYGVILTALFLLYCKRGRKKLLYIFKQPFMRPVQTTQEEDGCSCRFPEEEEGGCELGGGGSGGGGSGGGGSMQDEDGYMTLNVQSKKRSSAQTSQLTFKDYSVTLHWYKGSGEGRGSLLTCGDVEENPGPMALPVTALLLPLALLLHAARPNWVNVISDLKKIEDLIQSMHIDATLYTESDVHPSCKVTAMKCFLLELQVISLESGDASIHDTVENLIILANNSLSSNGNVTESGCKECEELEEKNIKEFLQSFVHIVQMFINTSTTTPAPRPPTPAPTIASQPLSLRPEACRPAAGGAVHTRGLDFACDIYIWAPLAGTCGVLLLSLVITLYC

SEQ ID NO: 21 - DNA, 1548 bp, Homo sapiens
  misc_feature: NK39-10 DNA
atggctctgcccgtcaccgcactgctgctgcctctggctctgctgctgcacgccgcacgaccactgttcaatcaggaagtccagatccccctgacagagtcttactgcggcccatgtcccaagaactggatctgctacaagaacaattgttatcagttctttgacgagagcaagaactggtatgagtcccaggcctcttgcatgagccagaatgcctctctgctgaaggtgtacagcaaggaggaccaggatctgctgaagctggtgaagtcctatcactggatgggcctggtgcacatccctacaaacggctcttggcagtgggaggacggctccatcctgtctccaaatctgctgaccatcatcgagatgcagaagggcgattgcgccctgtacgccagctccttcaagggctatatcgagaactgctccacacccaatacctacatctgtatgcagaggaccgtgaccacaacccctgcaccacgcccccctacaccagcacctaccatcgcaagccagcctctgtccctgcggccagaggcatgtagaccagcagcaggaggagcagtgcacacaagaggcctggacttcgcctgcgatcccaaactctgctacctgctggatggaatcctcttcatctatggtgtcattctcactgccttgttcctgaagacaaatatcaggtctagcacccgcgactggaaggatcacaagtttaagtggcggaaggaccctcaggataagaagcggggcagaaagaagctgctgtatatcttcaagcagcccttcatgcggcccgtgcagacaacccaggaggaagacggctgctcatgtagatttcctgaagaagaagaagggggctgtgaactgggctctggcgagggaaggggttccctgcttacttgcggcgacgtcgaagagaatcccggtccgatggccctcccagtaactgccctccttttgcccctcgcactccttcttcatgccgctcgccccaactgggtcaacgtgattagcgatttgaagaaaatcgaggaccttatacagtctatgcatattgacgctacactgtatactgagagtgatgtacacccgtcctgtaaggtaacggccatgaaatgctttcttctggagctccaggtcatcagcttggagtctggggacgcaagcatccacgatacggttgaaaacctcatcatccttgcgaacaactctctctcatctaatggaaacgttacagagagtgggtgtaaggagtgcgaagagttggaagaaaaaaacatcaaagaatttcttcaatccttcgttcacatagtgcaaatgttcattaacacgtccactaccacacccgccccgaggccacctacgccggcaccgactatcgccagtcaacccctctctctgcgccccgaggcttgccggcctgcggctggtggggcggtccacacccggggcctggattttgcgtgcgatatatacatctgggcacctcttgccggcacctgcggagtgctgcttctctcactcgttattacgctgtactgc

SEQ ID NO: 22 - protein, 516 aa, Homo sapiens
  MISC_FEATURE: NK39-109 Amino Acid
MALPVTALLLPLALLLHAARPLFNQEVQIPLTESYCGPCPKNWICYKNNCYQFFDESKNWYESQASCMSQNASLLKVYSKEDQDLLKLVKSYHWMGLVHIPTNGSWQWEDGSILSPNLLTIIEMQKGDCALYASSFKGYIENCSTPNTYICMQRTVTTTPAPRPPTPAPTIASQPLSLRPEACRPAAGGAVHTRGLDFACDPKLCYLLDGILFIYGVILTALFLKTNIRSSTRDWKDHKFKWRKDPQDKKRGRKKLLYIFKQPFMRPVQTTQEEDGCSCRFPEEEEGGCELGSGEGRGSLLTCGDVEENPGPMALPVTALLLPLALLLHAARPNWVNVISDLKKIEDLIQSMHIDATLYTESDVHPSCKVTAMKCFLLELQVISLESGDASIHDTVENLIILANNSLSSNGNVTESGCKECEELEEKNIKEFLQSFVHIVQMFINTSTTTPAPRPPTPAPTIASQPLSLRPEACRPAAGGAVHTRGLDFACDIYIWAPLAGTCGVLLLSLVITLYC

SEQ ID NO: 23 - DNA, 645 bp, Homo sapiens
  misc_feature: Full length human NKG2D
gggtggattcgtggtcggaggtctcgacacagctgggagatgagtgaatttcataattataacttggatctgaagaagagtgatttttcaacacgatggcaaaagcaaagatgtccagtagtcaaaagcaaatgtagagaaaatgcatctccattttttttctgctgcttcatcgctgtagccatgggaatccgtttcattattatggtaacaatatggagtgctgtattcctaaactcattattcaaccaagaagttcaaattcccttgaccgaaagttactgtggcccatgtcctaaaaactggatatgttacaaaaataactgctaccaattttttgatgagagtaaaaactggtatgagagccaggcttcttgtatgtctcaaaatgccagccttctgaaagtatacagcaaagaggaccaggatttacttaaactggtgaagtcatatcattggatgggactagtacacattccaacaaatggatcttggcagtgggaagatggctccattctctcacccaacctactaacaataattgaaatgcagaagggagactgtgcactctatgcctcgagctttaaaggctatatagaaaactgttcaactccaaatacgtacatctgcatgcaaaggactgtg

SEQ ID NO: 24 - DNA, 405 bp, Homo sapiens
  misc_feature: Truncated human NKG2D DNA
ttattcaaccaagaagttcaaattcccttgaccgaaagttactgtggcccatgtcctaaaaactggatatgttacaaaaataactgctaccaattttttgatgagagtaaaaactggtatgagagccaggcttcttgtatgtctcaaaatgccagccttctgaaagtatacagcaaagaggaccaggatttacttaaactggtgaagtcatatcattggatgggactagtacacattccaacaaatggatcttggcagtgggaagatggctccattctctcacccaacctactaacaataattgaaatgcagaagggagactgtgcactctatgcctcgagctttaaaggctatatagaaaactgttcaactccaaatacgtacatctgcatgcaaaggactgtg

SEQ ID NO: 25 - DNA, 405 bp, Homo sapiens
  misc_feature: Codon optimized truncated human NKG2D DNA
ctgttcaatcaggaagtccagatccccctgacagagtcttactgcggcccatgtcccaagaactggatctgctacaagaacaattgttatcagttctttgacgagagcaagaactggtatgagtcccaggcctcttgcatgagccagaatgcctctctgctgaaggtgtacagcaaggaggaccaggatctgctgaagctggtgaagtcctatcactggatgggcctggtgcacatccctacaaacggctcttggcagtgggaggacggctccatcctgtctccaaatctgctgaccatcatcgagatgcagaagggcgattgcgccctgtacgccagctccttcaagggctatatcgagaactgctccacacccaatacctacatctgtatgcagaggaccgtg

SEQ ID NO: 26 - DNA, 135 bp, Homo sapiens
  misc_feature: CD8a hinge
accacaacccctgcaccacgcccccctacaccagcacctaccatcgcaagccagcctctgtccctgcggccagaggcatgtagaccagcagcaggaggagcagtgcacacaagaggcctggacttcgcctgcgat

SEQ ID NO: 27 - DNA, 72 bp, Homo sapiens
  misc_feature: CD8a TM domain
atatacatctgggcacctcttgccggcacctgcggagtgctgcttctctcactcgttattacgctgtactgc

SEQ ID NO: 28 - protein, 12 aa, Homo sapiens
  MISC_FEATURE: Ig4 Short hinge protein
ESKYGPPCPSCP

SEQ ID NO: 29 - DNA, 87 bp, Homo sapiens
  misc_feature: CD28 TM Domain
ttttgggtgctggtggtggttggtggagtcctggcttgctatagcttgctagtaacagtggcctttattattttctgggtgaggagt

SEQ ID NO: 30 - DNA, 69 bp, Homo sapiens
  misc_feature: CD3 TM Domain
cccaaactctgctacctgctggatggaatcctcttcatctatggtgtcattctcactgccttgttcctg

SEQ ID NO: 31 - DNA, 126 bp, Homo sapiens
  misc_feature: 4-1BB Domain
aaacggggcagaaagaaactcctgtatatattcaaacaaccatttatgagaccagtacaaactactcaagaggaagatggctgtagctgccgatttccagaagaagaagaaggaggatgtgaactg

SEQ ID NO: 32 - DNA, 336 bp, Homo sapiens
  misc_feature: CD3zeta ITAM
agagtgaagttcagcaggagcgcagacgcccccgcgtaccagcagggccagaaccagctctataacgagctcaatctaggacgaagagaggagtacgatgttttggacaagagacgtggccgggaccctgagatggggggaaagccgagaaggaagaaccctcaggaaggcctgtacaatgaactgcagaaagataagatggcggaggcctacagtgagattgggatgaaaggcgagcgccggaggggcaaggggcacgatggcctttaccagggtctcagtacagccaccaaggacacctacgacgcccttcacatgcaggccctgccccctcgc

SEQ ID NO: 33 - DNA, 336 bp, Homo sapiens; identical to SEQ ID NO: 32
  misc_feature: CD3z no ITAM

SEQ ID NO: 34 - DNA, 117 bp, Homo sapiens
  misc_feature: CD29 signalling Domain
aagaggagcaggctcctgcacagtgactacatgaacatgactccccgccgccccgggcccacccgcaagcattaccagccctatgccccaccacgcgacttcgcagcctatcgctcc

SEQ ID NO: 35 - DNA, 111 bp, Homo sapiens
  misc_feature: OX-40 Domain
cggagggaccagaggctgccccccgatgcccacaagccccctgggggaggcagtttccggacccccatccaagaggagcaggccgacgcccactccaccctggccaagatc

SEQ ID NO: 36 - DNA, 114 bp, Homo sapiens
  misc_feature: NKp80 Domain
atgcaggatgaggacggctacatgaccctgaacgtgcagagcaagaagaggagcagcgcccagaccagccagctgaccttcaaggactacagcgtgaccctgcactggtacaag

SEQ ID NO: 37 - DNA, 75 bp, Homo sapiens
  misc_feature: CD16 IC Domain
aagacaaatatcaggtctagcacccgcgactggaaggatcacaagtttaagtggcggaaggaccctcaggataag

SEQ ID NO: 38 - DNA, 63 bp, Homo sapiens
  misc_feature: 2A Stop
ggctctggcgagggaaggggttccctgcttacttgcggcgacgtcgaagagaatcccggtccg

SEQ ID NO: 39 - DNA, 614 bp, Homo sapiens
  misc_feature: mbIL-15
atggccttaccagtgaccgccttgctcctgccgctggccttgctgctccacgccgccaggccgaactgggtgaatgtaataagtgatttgaaaaaaattgaagatcttattcaatctatgcatattgatgctactttatatacggaaagtgatgttcaccccagttgcaaagtaacagcaatgaagtgctttctcttggagttacaagttatttcacttgagtccggagatgcaagtattcatgatacagtagaaaatctgatcatcctagcaaacaacagtttgtcttctaatgggaatgtaacagaatctggatgcaaagaatgtgaggaactggaggaaaaaaatattaaagaatttttgcagagttttgtacatattgtccaaatgttcatcaacacttctaccacgacgccagcgccgcgaccaccaacaccggcgcccaccatcgcgtcgcagcccctgtccctgcgcccagaggcgtgccggccagcggcggggggcgcagtgcacacgagggggctggacttcgcctgtgatatctacatctgggcgcccttggccgggacttgtggggtccttctcctgtcactggtatcaccctttactgctaa

SEQ ID NO: 40 - DNA, 117 bp, Homo sapiens; identical to SEQ ID NO: 34
  misc_feature: CD28 Signalling Domain

SEQ ID NO: 41 - protein, 15 aa, Homo sapiens
  MISC_FEATURE: GS3 Linker
GGGGSGGGGSGGGGS

SEQ ID NO: 42 - protein, 8 aa, Homo sapiens
  MISC_FEATURE: FLAG Tag
DYKDDDDK

SEQ ID NO: 43 - protein, 6 aa, Homo sapiens
  MISC_FEATURE: HIS Tag
HHHHHH

SEQ ID NO: 44 - protein, 10 aa, Homo sapiens
  MISC_FEATURE: Myc Tag
EQKLISEEDL